European Patent Application EP 4 166 569 A1, published April 19, 2023. Title: ANTIBODIES DIRECTED AGAINST ALPHA-FOLATE RECEPTOR. Applicant: Fondazione IRCCS Istituto Nazionale dei Tumori. The sequence listing filed with the application follows.

SEQUENCE LISTING (14 sequences)

SEQ ID NO: 1 - protein, 8 aa, Unknown
  VH CDR1
DYIFTNYD

SEQ ID NO: 2 - protein, 8 aa, Unknown
  VH CDR2
IDPRSGKS

SEQ ID NO: 3 - protein, 14 aa, Unknown
  VH CDR3
ATMYYYGSSPPMDY

SEQ ID NO: 4 - protein, 6 aa, Unknown
  VL CDR1
QDINNF

SEQ ID NO: 5 - skipped

SEQ ID NO: 6 - protein, 9 aa, Unknown
  VL CDR3
QQSSTIPRT

SEQ ID NO: 7 - protein, 123 aa, Unknown
  VH Mov18
QVQLQQSGAELARPGASVKLSCKASDYIFTNYDITWVKQRPGQGLEWIGEIDPRSGKSYYNEKFKGKSTLTADKSSSTAYMELRSLTSEDSAVYFCATMYYYGSSPPMDYWGQGTSVTVSRRE

SEQ ID NO: 8 - protein, 107 aa, Unknown
  VL Mov18
DIQMTQTTSSLSASLGDRVTISCRASQDINNFLNWYQQKPDGTVKLLIYYTSRLHSGVPSRFSGSGSGTDYSLTIINLEQEDIAIYFCQQSSTIPRTFGQGTKLEIK

SEQ ID NO: 9 - protein, 120 aa, Unknown
  VH Antibody I
QVQLVQSGSELKKPGASVKVSCKASDYIFTNYDITWVRQAPGQGLEWMGEIDPRSGKSYYNEKFKGKSTLTADKSVSTAYLQISSLKAEDTAVYFCATMYYYGSSPPMDYWGQGTTVTVS

SEQ ID NO: 10 - protein, 107 aa, Unknown
  VL Antibody I
DIQMTQSPSSLSASVGDRVTITCRASQDINNFLNWYQQKPGKAPKLLIYYTSRLHSGVPSRFSGSGSGTDYTFTISSLQPEDIATYFCQQSSTIPRTFGQGTKLEIK

SEQ ID NO: 11 - protein, 120 aa, Unknown
  VH Antibody II
QVQLVQSGSEVKKPGASVKVSCKASDYIFTNYDITWVRQAPGQGLEWMGEIDPRSGKSYYNEKFQGRSTLTADKSVSTAYLEISSLKAEDTAVYFCATMYYYGSSPPMDYWGQGTTVTVS

SEQ ID NO: 12 - protein, 107 aa, Unknown
  VL Antibody II
DIQMTQSPSSLSASVGDRVTITCQASQDINNFLNWYQQKPGKAPKLLIYYTSRLHSGVPSRFSGSGSGTDFTFTISSLQPEDIATYFCQQSSTIPRTFGQGTKLEIK

SEQ ID NO: 13 - DNA, 360 bp, Unknown
  VH Antibody I
caggtgcagctggtgcaatctgggtctgagttgaagaagcctggggcctcagtgaaagtttcctgcaaggctagcgactacatcttcactaactatgacataacctgggtgcgacaggcccctggccaggggcttgagtggatgggagagattgatcctaggagtggtaagagttattataatgagaaattcaagggcaagtccacactgactgcagacaaatctgtcagcacggcatatctgcagatcagcagcctaaaggctgaggacacggccgtgtatttctgtgcgacaatgtactactacggctcgagcccccctatggactactggggtcaaggaaccactgtcaccgtctcc

SEQ ID NO: 14 - DNA, 321 bp, Unknown
  VL Antibody I
gatatccagatgacccagagtccaagcagcctgagtgctagcgtgggagatcgcgtgaccatcacgtgtagggccagtcaggacattaacaattttttaaactggtaccagcagaagcctggtaaggctccaaagctgctgatctactacacctcgagattacactcaggagtgccatctcgcttcagcggttctggaagcggtaccgactataccttcaccatcagcagcctccagcctgaggatatcgctacgtacttctgtcaacagagtagtacgattcctaggacgttcggacagggaaccaagctggaaatcaag